European Patent Specification EP 4 540 411 B1, published May 13, 2026. Title: PROCEDE POUR L'INTEGRATION CIBLEE D'IDENTIFICATEURS MOLECULAIRES UNIQUES (IUM) ET LA DETECTION DE HAUTE PRECISION D'ETATS MEDICAUX OU COSMETIQUES. Applicant: GRAND HOPITAL DE CHARLEROI. Application BE BE2023/5056, filed January 30, 2023. The sequence listing filed with the application follows.

SEQUENCE LISTING (8 sequences)

SEQ ID NO: 1 - DNA, 62 bp, synthetic construct
  source 1..62: mol_type = other DNA
aagcagtggtatcaacgcagagtgcagnnnntnnntnnntagctggtgtggccttttgggtg

SEQ ID NO: 2 - DNA, 26 bp, synthetic construct
  source 1..26: mol_type = other DNA
atacttctattggtacagacaaatct

SEQ ID NO: 3 - DNA, 23 bp, synthetic construct
  source 1..23: mol_type = other DNA
aagcagtggtatcaacgcagagt

SEQ ID NO: 4 - DNA, 41 bp, synthetic construct
  source 1..41: mol_type = other DNA
aagactcggcagcatctccaactctgaagatccggtccaca

SEQ ID NO: 5 - DNA, 43 bp, synthetic construct
  source 1..43: mol_type = other DNA
gcgatcgtcactgttctccagcagtggtatcaacgcagagtgc

SEQ ID NO: 6 - DNA, 18 bp, synthetic construct
  source 1..18: mol_type = other DNA
gtgttcccacccgaggtc

SEQ ID NO: 7 - DNA, 43 bp, synthetic construct
  source 1..43: mol_type = other DNA
gtagcagaggatatcaacgcaagtannntnnntnnnnrgrgrg

SEQ ID NO: 8 - DNA, 43 bp, synthetic construct
  source 1..43: mol_type = other DNA
gcgatcgtcactgttctccatctctgcttctgatggctcaaac